European Patent Specification EP 4 074 337 B1, published May 7, 2025. Title: PHARMACEUTICAL TACI-FC FUSION PROTEIN FORMULATION. Applicant: REMEGEN CO., LTD. The sequence listing filed with the application follows.

SEQUENCE LISTING (1 sequence)

SEQ ID NO: 1 - protein, 333 aa, artificial sequence
  RC18 amino acid sequence
SRVDQEERFPQGLWTGVAMRSCPEEQYWDPLLGTCMSCKTICNHQSQRTCAAFCRSLSCRKEQGKFYDHLLRDCISCASICGQHPKQCAYFCENKLRSPVNLPPELDKTHTCPPCPAPEAEGAPSVFLFPPKPKDTLMISRTPEVTCVVVDVSHEDPEVKFNWYVDGVEVHNAKTKPREEQYNSTYRVVSVLTVLHQDWLNGKEYKCKVSNKALPSSIEKTISKAKGQPREPQVYTLPPSRDELTKNQVSLTCLVKGFYPSDIAVEWESNGQPENNYKTTPPVLDSDGSFFLYSKLTVDKSRWQQGNVFSCSVMHEALHNHYTQKSLSLSPGK